European Patent Specification EP 3 628 729 B1, published July 9, 2025. Title: Arrays, Substrates, Devices, Methods and Systems for Detecting Target Molecules. Applicant: CALIFORNIA INSTITUTE OF TECHNOLOGY. The sequence listing filed with the application follows.

SEQUENCE LISTING (41 sequences)

SEQ ID NO: 1 - DNA, 33 bp, artificial sequence
  Synthetic Polynucleotide
aaaaaaaaaaaaaatcctggagctaagtccgta

SEQ ID NO: 2 - DNA, 30 bp, artificial sequence
  Synthetic Polynucleotide
aaaaaaaaaatacggacttagctccaggat

SEQ ID NO: 3 - DNA, 33 bp, artificial sequence
  Synthetic Polynucleotide
aaaaaaaaaaaaagcctcattgaatcatgccta

SEQ ID NO: 4 - DNA, 30 bp, artificial sequence
  Synthetic Polynucleotide
aaaaaaaaaataggcatgattcaatgaggc

SEQ ID NO: 5 - DNA, 33 bp, artificial sequence
  Synthetic Polynucleotide
aaaaaaaaaaaaagcactcgtctactatcgcta

SEQ ID NO: 6 - DNA, 30 bp, artificial sequence
  Synthetic Polynucleotide
aaaaaaaaaatagcgatagtagacgagtgc

SEQ ID NO: 7 - DNA, 33 bp, artificial sequence
  Synthetic Polynucleotide
aaaaaaaaaaaaaatggtcgagatgtcagagta

SEQ ID NO: 8 - DNA, 30 bp, artificial sequence
  Synthetic Polynucleotide
aaaaaaaaaatactctgacatctcgaccat

SEQ ID NO: 9 - DNA, 33 bp, artificial sequence
  Synthetic Polynucleotide
aaaaaaaaaaaaaatgtgaagtggcagtatcta

SEQ ID NO: 10 - DNA, 30 bp, artificial sequence
  Synthetic Polynucleotide
aaaaaaaaaatagatactgccacttcacat

SEQ ID NO: 11 - DNA, 33 bp, artificial sequence
  Synthetic Polynucleotide
aaaaaaaaaaaaaatcaggtaaggttcacggta

SEQ ID NO: 12 - DNA, 30 bp, artificial sequence
  Synthetic Polynucleotide
aaaaaaaaaataccgtgaaccttacctgat

SEQ ID NO: 13 - DNA, 30 bp, artificial sequence
  Synthetic Polynucleotide
aaaaaaaaaagagtagccttcccgagcatt

SEQ ID NO: 14 - DNA, 30 bp, artificial sequence
  Synthetic Polynucleotide
aaaaaaaaaaaatgctcgggaaggctactc

SEQ ID NO: 15 - DNA, 30 bp, artificial sequence
  Synthetic Polynucleotide
aaaaaaaaaaattgaccaaactgcggtgcg

SEQ ID NO: 16 - DNA, 30 bp, artificial sequence
  Synthetic Polynucleotide
aaaaaaaaaacgcaccgcagtttggtcaat

SEQ ID NO: 17 - DNA, 30 bp, artificial sequence
  Synthetic Polynucleotide
aaaaaaaaaatgccctattgttgcgtcgga

SEQ ID NO: 18 - DNA, 30 bp, artificial sequence
  Synthetic Polynucleotide
aaaaaaaaaatccgacgcaacaatagggca

SEQ ID NO: 19 - DNA, 29 bp, artificial sequence
  Synthetic Polynucleotide
aaaaaaaaatcttctagttgtcgagcagg

SEQ ID NO: 20 - DNA, 30 bp, artificial sequence
  Synthetic Polynucleotide
aaaaaaaaaacctgctcgacaactagaaga

SEQ ID NO: 21 - DNA, 30 bp, artificial sequence
  Synthetic Polynucleotide
aaaaaaaaaataatctaattctggtcgcgg

SEQ ID NO: 22 - DNA, 30 bp, artificial sequence
  Synthetic Polynucleotide
aaaaaaaaaaccgcgaccagaattagatta

SEQ ID NO: 23 - DNA, 30 bp, artificial sequence
  Synthetic Polynucleotide
aaaaaaaaaagtgattaagtctgcttcggc

SEQ ID NO: 24 - DNA, 30 bp, artificial sequence
  Synthetic Polynucleotide
aaaaaaaaaagccgaagcagacttaatcac

SEQ ID NO: 25 - DNA, 30 bp, artificial sequence
  Synthetic Polynucleotide
aaaaaaaaaagtcgaggattctgaacctgt

SEQ ID NO: 26 - DNA, 30 bp, artificial sequence
  Synthetic Polynucleotide
aaaaaaaaaaacaggttcagaatcctcgac

SEQ ID NO: 27 - DNA, 30 bp, artificial sequence
  Synthetic Polynucleotide
aaaaaaaaaagtcacagactagccacgaag

SEQ ID NO: 28 - DNA, 30 bp, artificial sequence
  Synthetic Polynucleotide
aaaaaaaaaagcgtgtgtggactctctcta

SEQ ID NO: 29 - DNA, 30 bp, artificial sequence
  Synthetic Polynucleotide
aaaaaaaaaatagagagagtccacacacgc

SEQ ID NO: 30 - DNA, 30 bp, artificial sequence
  Synthetic Polynucleotide
aaaaaaaaaatcttctagttgtcgagcagg

SEQ ID NO: 31 - DNA, 30 bp, artificial sequence; identical to SEQ ID NO: 20
  Synthetic Polynucleotide

SEQ ID NO: 32 - DNA, 30 bp, artificial sequence
  Synthetic Polynucleotide
aaaaaaaaaagatcgtatggtccgctctca

SEQ ID NO: 33 - DNA, 30 bp, artificial sequence
  Synthetic Polynucleotide
aaaaaaaaaatgagagcggaccatacgatc

SEQ ID NO: 34 - DNA, 30 bp, artificial sequence
  Synthetic Polynucleotide
aaaaaaaaaagcactaactggtctgggtca

SEQ ID NO: 35 - DNA, 30 bp, artificial sequence
  Synthetic Polynucleotide
aaaaaaaaaatgacccagaccagttagtgc

SEQ ID NO: 36 - DNA, 30 bp, artificial sequence; identical to SEQ ID NO: 17
  Synthetic Polynucleotide

SEQ ID NO: 37 - DNA, 30 bp, artificial sequence; identical to SEQ ID NO: 18
  Synthetic Polynucleotide

SEQ ID NO: 38 - DNA, 30 bp, artificial sequence
  Synthetic Polynucleotide
aaaaaaaaaactctgtgaactgtcatcggt

SEQ ID NO: 39 - DNA, 30 bp, artificial sequence
  Synthetic Polynucleotide
aaaaaaaaaaaccgatgacagttcacagag

SEQ ID NO: 40 - DNA, 30 bp, artificial sequence; identical to SEQ ID NO: 13
  Synthetic Polynucleotide

SEQ ID NO: 41 - DNA, 30 bp, artificial sequence; identical to SEQ ID NO: 14
  Synthetic Polynucleotide